European Patent Application EP 4 257 188 A1, published October 11, 2023. Title: DERMATOLOGISCH WIRKSAME ZUSAMMENSETZUNG MIT CATECHINEN UND FLAVONOIDEN. Applicant: BioActive Food GmbH. The sequence listing filed with the application follows.

SEQUENCE LISTING (18 sequences)

SEQ ID NO: 1 - DNA, 20 bp, Artificial Sequence
  Primer
aattgaggctgagccaaaga

SEQ ID NO: 2 - DNA, 21 bp, Artificial Sequence
  Primer
tgtccatcaagtgaaccccag

SEQ ID NO: 3 - DNA, 21 bp, Artificial Sequence
  Primer
ctggaagagtggagagtactg

SEQ ID NO: 4 - DNA, 20 bp, Artificial Sequence
  Primer
gtctccatgttgcagaagac

SEQ ID NO: 5 - DNA, 24 bp, Artificial Sequence
  Primer
ggcaaatcctgaagaatccagatg

SEQ ID NO: 6 - DNA, 26 bp, Artificial Sequence
  Primer
ggtaaattctcttttctggtagactc

SEQ ID NO: 7 - DNA, 20 bp, Artificial Sequence
  Primer
gttccccagaaactgtggga

SEQ ID NO: 8 - DNA, 19 bp, Artificial Sequence
  Primer
cgagacgttctgcagaacc

SEQ ID NO: 9 - DNA, 21 bp, Artificial Sequence
  Primer
ggaggaggaacagtcttgagg

SEQ ID NO: 10 - DNA, 20 bp, Artificial Sequence
  Primer
ctgcctcagccttactgtga

SEQ ID NO: 11 - DNA, 21 bp, Artificial Sequence
  Primer
ctctcctcactcacccttcct

SEQ ID NO: 12 - DNA, 19 bp, Artificial Sequence
  Primer
aggtcttcacgcagtccac

SEQ ID NO: 13 - DNA, 22 bp, Artificial Sequence
  TCAAGGACTTCCTGCTCACA
aacaatggtcatgctttcaacg

SEQ ID NO: 14 - DNA, 21 bp, Artificial Sequence
  Primer
tgtccatcaagtgaaccccag

SEQ ID NO: 15 - DNA, 20 bp, Artificial Sequence
  Primer
tcaaggacttcctgctcaca

SEQ ID NO: 16 - DNA, 21 bp, Artificial Sequence
  Primer
aaaggtatctgctgcatcgaa

SEQ ID NO: 17 - DNA, 15 bp, Artificial Sequence
  Primer
ggaagcggcccgtgt

SEQ ID NO: 18 - DNA, 17 bp, Artificial Sequence
  Primer
ccaggctgactggcacg